European Patent Application EP 4 382 617 A1, published June 12, 2024. Title: 一种肿瘤评估方法及应用. Applicant: 江苏鹍远生物技术有限公司. The sequence listing filed with the application follows.

SEQUENCE LISTING (139 sequences)

SEQ ID NO: 1 - DNA, 2070 bp, synthetic construct
  misc_feature 1..2070: note = SEPT9(1) subregion
  source 1..2070: mol_type = other DNA
cctgctctcaggaggcccttattgtggaggaagggaggcgtcgcccgtccctggcttctctgacagccgtgttccatccccgccctgtgccccttctcccggacagtgccttctccagggctcacccaggagggtgcagcggtggcccccggggcggtggtcgtggtgggggtgttagctgcaggggtgccctcggtgggtgggagttggtggcctctcgctggtgccatgggactcgcatgttcgccctgcgcccctcggctcttgagcccacaggccgggatcctgcctgccagccgcgtgcgctgccgtttaacccttgcaggcgcagagcgcgcggcggcggtgacagagaactttgtttggctgcccaaatacagcctcctgcagaaggaccctgcgcccggggaaggggaggaatctcttcccctctgggcgcccgccctcctcgccatggcccggcctccacatccgcccacatctggccgcagcggggcgcccggggggaggggctgaggccgcgtctctcgccgtcccctgggcgcgggccaggcggggaggaggggggcgctccggtcgtgtgcccaggactgtcccccagcggccactcgggccccagccccccaggcctggccttgacaggcgggcggagcagccagtgcgagacagggaggccggtgcgggtgcgggaacctgatccgcccgggaggcgggggcggggcgggggcgcagcgcgcggggaggggccggcgcccgccttcctcccccattcattcagctgagccagggggcctaggggctcctccggcggctagctctgcactgcaggagcgcgggcgcggcgccccagccagcgcgcagggcccgggccccgccgggggcgcttcctcgccgctgccctccgcgcgacccgctgcccaccagccatcatgtcggaccccgcggtcaacgcgcagctggatgggatcatttcggacttcgaaggtgggtgctgggctggctgctgcggccgcggacgtgctggagaggaccctgcgggtgggcctggcgcgggacgggggtgcgctgaggggagacgggagtgcgctgaggggagacgggacccctaatccaggcgccctcccgctgagagcgccgcgcgcccccggccccgtgcccgcgccgcctacgtgggggaccctgttaggggcacccgcgtagaccctgcgcgccctcacaggaccctgtgctcgttctgcgcactgccgcctgggtttccttccttttattgttgtttgtgtttgccaagcgacagcgacctcctcgagggctcgcgaggctgcctcggaactctccaggacgcacagtttcactctgggaaatccatcggtcccctccctttggctctccccggcggctctcgggccccgcttggacccggcaacgggatagggaggtcgttcctcacctccgactgagtggacagccgcgtcctgctcgggtggacagccctcccctcccccacgccagtttcggggccgccaagttgtgcagcccgtgggccgggagcaccgaacggacacagcccaggtcgtggcagggtctagagtgggatgtcccatggcccccatccaggcctggggatatcctcatccgcctcccagaatcgggccgtgggggacagaaggggcctgcgtgcgggcagggagagtattttggctctctcctgtcttcggggtttacaaagtgtgttgggacttgcggggctgctctgtccaagcctgggtctggcgtccgcgtctctgagcctgtgagtgcgtgcgctttcctgcgtcctcttgactgccggtgctggggctctgcgtcctgcgtccgcgggagtaaatacagcaggcgaaggggaagctcacacaatggtctccagcgctctggggcagggcttctgaggggcgggcctgcctctgccgggacctggagcccccgcccctcggagaggctcctaggctgacttgggcagagccctctggtgggccgggagggggaaaggctgtgttgaaatgagcaaactgtccaggtgtcaggccaagctgg

SEQ ID NO: 2 - DNA, 18 bp, synthetic construct
  misc_feature 1..18: note = SEPT9(1) probe
  source 1..18: mol_type = other DNA
ttaaccgcgaaatccgac

SEQ ID NO: 3 - DNA, 19 bp, synthetic construct
  misc_feature 1..19: note = SEPT9(1) forward primer
  source 1..19: mol_type = other DNA
aaataatcccatccaacta

SEQ ID NO: 4 - DNA, 26 bp, synthetic construct
  misc_feature 1..26: note = SEPT9(1) reverse primer
  source 1..26: mol_type = other DNA
gattcgttgtttattagttattatgt

SEQ ID NO: 5 - DNA, 828 bp, synthetic construct
  misc_feature 1..828: note = IKZF1 subregion
  source 1..828: mol_type = other DNA
gcacccgccgccgccccggcggcctttgggggctgagccggagcccggcgcgattgcaaagttttcgtgcgcggcccctctggcccggagttgcggctgagacgcgcgccgcgcgagccgggggactcggcgacggggcggggacgggacgacgcaccctctccgtgtcccgctctgcgcccttctgcgcgccccgctccctgtaccggagcagcgatccgggaggcggccgagaggtgcgcgcggggccgagccggctgcggggcaggtcgagcagggaccgccagcgtgcgtcaccccaaagtttgcggggtggcagggcgcgcgctctggccacccgccgctctgggcggcagctggtggcaacgcaagggcgcggcgggggcggccggcgcggagggggccaggtacggggcccgcgggcggcgctgtgcgcgcggggcagccggtcggccgggagcgcgaaagcctggtctgagccggctgggggcggggagtgtggcggagaaatggggaacaatgcgagtgagcaacttcaggaagtcattgtgaaagaaagctgggaagagctccgcggccaagttagcaggacactctaacaagtgactgcgcggcccgcgcccggggcggtgactgcggcaagccccctgggtccccgcgcggcgcatcccagcctgggcgggacgctcggccgcggcgaggcgggcaagcctggcagggcagagggagccccggctccgaggttgctcttcgcacccgaggatcagtcttggccccaaagcgcgacgcacaaatccacgtgagtgttttcaaattgaatttcaatag

SEQ ID NO: 6 - DNA, 16 bp, synthetic construct
  misc_feature 1..16: note = IKZF1 probe
  source 1..16: mol_type = other DNA
cgccccgtcgccgaat

SEQ ID NO: 7 - DNA, 20 bp, synthetic construct
  misc_feature 1..20: note = IKZF1 forward primer
  source 1..20: mol_type = other DNA
gtttttttggttcggagttg

SEQ ID NO: 8 - DNA, 23 bp, synthetic construct
  misc_feature 1..23: note = IKZF1 reverse primer
  source 1..23: mol_type = other DNA
caaaacgaaacacgaaaaaaata

SEQ ID NO: 9 - DNA, 750 bp, synthetic construct
  misc_feature 1..750: note = BEST4 subregion
  source 1..750: mol_type = other DNA
cacgattcaactggcctggaccaggccctttgctgggggaggtgaggcgctccgacccccaggctctccactctcccttcctactccctctatcacggcggccaagcaggtttctatgtgactctcgtggtgaaccgctggtggtcccagtacacaagcatcccgctgccagaccagctgatgtgcgtcatctcggctagcgtgcacggcgtggaccagcggggccgcctgctgcgccgcaccctcatccgctacgcgaacctggcgtccgtgctggtgctgcgctcggtcagcacccgcgtgcttaagcgcttccccaccatggagcacgtggtggacgcaggtgcgccgcccgccgggagcctctgggggtccggcccacagccggatgcaggtggcgcctgggagagtcctgggagcaggggcctccagggaagggtctggactgcgacaggaacgcggaaccgcgagtcctgggacagccggtggacgcgagggaggggagccagacggcggaacagcagcctcccctggcggcagagggtgcaactgcaccccacctgctttaccccctcaggtttcatgtcccaggaagagaggaaaaagtttgagagcctgaaatccgacttcaacaagtactgggtcccctgcgtctggttcaccaacctggcggcccaggcccggagggacgggcgaatacgtgacgatatcgctctctgtctacttttggaagtgagtgggctcaggacc

SEQ ID NO: 10 - DNA, 23 bp, synthetic construct
  misc_feature 1..23: note = BEST4 probe
  source 1..23: mol_type = other DNA
cggcgtatttgcgtttattacgt

SEQ ID NO: 11 - DNA, 20 bp, synthetic construct
  misc_feature 1..20: note = BEST4 forward primer
  source 1..20: mol_type = other DNA
tgtgggtcggatttttagag

SEQ ID NO: 12 - DNA, 19 bp, synthetic construct
  misc_feature 1..19: note = BEST4 reverse primer
  source 1..19: mol_type = other DNA
tacttaaacgcttccccac

SEQ ID NO: 13 - DNA, 2465 bp, synthetic construct
  misc_feature 1..2465: note = B4GALNT1 subregion
  source 1..2465: mol_type = other DNA
ttcagggtcaaatgccatgtcctttcttcccagtccggttctccaccgagggacatgaggctgctttcactatccgcataagacacccgcccaaccctcggctgtacccacctgggtctctaccccagggaggtgaggctggtaggggcagggacatattagaaccagccttggtggggagcaagttgggagagggcagtcctgggaggggatatctacctgttcccctctcccaaccctccttgtctgcacccaaccctgtgcccccaatctcagcccagtacaacatcagcgctctagtcacgattgccaccaagaccttcctccgttatgatcggctacgggctctcatcaccagtatccgccgcttctacccaacggttaccgtggtcatcgctgacgacagcgacaagccagagcgcgttagtggcccctacgtggaacactatctcatgcccttcggcaaggtgtgcagctagcaggctgaacggcaggccagaggactcccgcagggggtgtgccctcaatctgcagcctccagggtagtgattcgaggaccacctgcctcagaatcatggggtgcctgttaagcatgaggattcctggaatgtaagcttcgtgggagcaggaaattctctctgaattcttagaatggtgcttagtgcctaatggcattcaataaaatagctgatgaatgaataaataaatgcacacggaaattaaacgcattctaagaccactgacttggaacctctgtggggatctgcatttcttttacctagctcctggcctttcgaaagcactcaaaagtctggagaagaatacaagctgagaagggtcgggggagagaaagaaaggtggcagagggccatgtcctatttctgcagcctccccaaccacacacacctttctgccagggctggttcgcaggccggaacctggccgtgtctcaagtaaccaccaagtacgtgctgtgggtggacgacgacttcgtcttcacggcgcggacgcggctggagaggcttgtggacgtgctggagcggacgccgctggacctggtagggcaggggctgcaggatgtgggggtggagaagggccttgaacaggctaaggccacagcgggggcgctgcggccaggaacggccagccctaggacaaagagagaaccacgaagtggggcctgggaactgtctgggtcctgcaggggtgaagcggaagaggatggggcaggggtacccccgaaggcaccggagcgcagaccttgaccccttcgggtcccctatcccaggcccgcctggaggcaacctccctctccctgcaggtggggggcgcggtgcgcgagatctccggctttgccaccacttatcggcagctgctgagcgtggagcccggcgccccaggcctcgggaactgcctccggcaaaggcgcggcttccaccacgagctcgtcggcttcccaggctgcgtggtcaccgacggcgtggttaacttcttcctggcgcggactgacaaggtgcgcgaggtcggtttcgacccccgcctcagccgcgtggctcatctgggtgagtggcaccccctcccggtcgaccctggcaggagccccacggggagctggcgcacggtcacgcgcctctcctcctaggctgcacccgcgcccagccgccagcgggaaccccagaacagttctgcagtgatttaccaagacctgcacctgggcgagagacagctcccaccctctcccagccccgcatactctttttttttttttataaatatatatattttttgttatactttaagttctagggtacatgtgcacaacgtgcaggtttgttacatgtgtatacatgtgccatgttgaatctccattcccagcacagccgctgggcccccataagcttccccatcactgttcccgccacccctgctctactcccagggcttcccctagttcagaccacagtcggtgcaacccatctggcgtttatttaacctctgggagtaggggtaggtttttcgattttcaaagcacaagtatattgactccatttacacaagagtaagactgagacccagggagttgatttacatgctcagggtccttagaaacaagcctttgcacacacactttccacaccctaaatttgagagttctcccttaccagtcggccttctgcaccctcaggatccctcactgtgtactcccctccacccccagaattcttcttggatgggcttggttcccttcgggttggctcctgctccgacgtcgtggtggatcatgcatccaaactgaagctgccttggacatcaagggatgccggagcagagacttacgcccggtaccgttacccaggatcactggacgagagccagatggccaaacaccggctgctcttcttcaaacaccggctgcagtgcatgacctcccagtgatggcccgctggggatttctgactgtcagg

SEQ ID NO: 14 - DNA, 21 bp, synthetic construct
  misc_feature 1..21: note = B4GALNT1 probe
  source 1..21: mol_type = other DNA
agatttcgcgtatcgcgtttt

SEQ ID NO: 15 - DNA, 20 bp, synthetic construct
  misc_feature 1..20: note = B4GALNT1 forward primer
  source 1..20: mol_type = other DNA
agtagttgtcgataagtggt

SEQ ID NO: 16 - DNA, 19 bp, synthetic construct
  misc_feature 1..19: note = B4GALNT1 reverse primer
  source 1..19: mol_type = other DNA
gcctaaaaacaacctccct

SEQ ID NO: 17 - DNA, 975 bp, synthetic construct
  misc_feature 1..975: note = GRASP subregion
  source 1..975: mol_type = other DNA
ccggctggcatcccccagccgccgccagccccgccgaggggagccagcgccgtctctgaggggcgtccggcgccggagccatgaccctccgccgactcaggaagctgcagcagaaggaggaggcggcggccaccccggaccccgccgcccggactcccgactcggaagtcgcgcccgccgctccggtcccgaccccgggaccccctgccgcagccgccacccctgggcccccagcggacgagctgtacgcggcgctggaggactatcaccctgccgagctgtaccgcgcgctcgccgtgtccgggggcaccctgccccgccgaaaggtgcgtcccccgcccgccttcaggatctgctcagcccctctccgactccctacagggcctgctgactccgcagtgccctctcctcggcgtccgcggagtcccccaccttcttccccggcccgctgggtgcctcgactccccgcgttccccgctgctgcgaaggccgtggccctcgcctgcacaccgcgcccaggctcggtggctcttaactccgcgccccatgcacgccccctctctccctccttgactcctcccagcaccccccttctcctacccgctccatctggctttctgccccccatgccccgcctccccgtggccaggtgtcctgggtccccaggagcccctcgcccgagggacagagacagccccaggcaagttgaaggtccgagagcccccggtgggagaagcgggccggtggctgcgccgcgtgcgttctcactctgaggaagtgcgtggggagccgctgactccggatagcacacccttccgaggggactccccgattcctgggctgggggcctgccgcctggccccacgtctgacgtacggggcgcgagggccactgctccctggacttctgtcggaaccggacgcagtgggaggggtcgcagggcgcccgcggggcaggaaggatgcgggccgcgcc

SEQ ID NO: 18 - DNA, 22 bp, synthetic construct
  misc_feature 1..22: note = GRASP probe
  source 1..22: mol_type = other DNA
tgtttttttttcggcgttcgcg

SEQ ID NO: 19 - DNA, 24 bp, synthetic construct
  misc_feature 1..24: note = GRASP forward primer
  source 1..24: mol_type = other DNA
gttttttttcgattttttataggg

SEQ ID NO: 20 - DNA, 25 bp, synthetic construct
  misc_feature 1..25: note = GRASP reverse primer
  source 1..25: mol_type = other DNA
aaccgaaaaaaaaaataaaaaactc

SEQ ID NO: 21 - DNA, 2318 bp, synthetic construct
  misc_feature 1..2318: note = IRF4 subregion
  source 1..2318: mol_type = other DNA
acctcgcactctcagtttcaccgctcgatcttgggacccaccgctgccctcagctccgagtccagggcgaggtaagggctggagtcgggcaggaggaggggtgtgaggctgataccagagaggacccggagcgcgaaccagaggttcgacctccagggcagcgcagggtaccccggcttcggagcgggaagggagcgcgccccgtcctggagctccgactcccaccccatctgcgctgagccggaggcgctggtttgggctccaaggcccgcctccttggctctgcccgagcctccccgcctgccctccgcgctcctgcgacggggtcgccacaagctggacgggatgagctaaccggactgtcggggccccaggagtggctgaggcggggccgtccaaggcacccacacaagacggcacaactgcctgcgagaaacaggcccggccctgtggaccccaatccgaggctccttcccctgctcttcgttcctaaggggcccaagctcacggcggcctccggcgcggtgctcacccgctggcgcaggaggaggaggagctccacatttgggtcgctccgagccttgcgtgcggtggcctagccggcctggcgcggtccctgcctcccaggctccgcagctgtcgtcgccctctcccgcgccctccccgcctccgctctcccgggcctgctccggggtccggcggacgctctgcgcgcggaatcccccgtactggggctgcagcccccgcgtctgcgccacttgtcgtttgcagagcccacttagtgcgcgctagctgggcagggataggggtcctattcggggcgaagggtctggatgcgagcagagaaagcggagggtggaggaacccggggctgcgcccctggaacgcccggccgcaggcgaggtcctccgcgcgtggaggccgccaggggagtggaaactgacagagtcgcggggaaggggcgagaagcgggttgggagtgagcgaaggcaagcgagagctgcgagtgagtgcggaaggagggccaggaggggtggcggctgggtggggagagagggtgcaagacgagcggcgcgtgtcgggagcctttgggctgcgggtgcgttacaggagagcaggcgggtaggagccttcgcgggggccgagctcggaaggcggacggctgtgcccgcccaggggatgcgcccgggccggccgcgaaggtgccttcttccgggggcccggacgaccctgacacggcacgcgcgcgcttcgcagcctcaaagactccggggcctcgtggtcactggcgcaggggatcggggcggggtgcccggagtgcggtgcctcgtggctgaagggcagctcttctccccgcagtgcagagcagagcgggcggaggaccccgggcgcgggcgcggacggcacgcggggcatgaacctggagggcggcggccgaggcggagagttcggcatgagcgcggtgagctgcggcaacgggaagctccgccagtggctgatcgaccagatcgacagcggcaagtaccccgggctggtgtgggagaacgaggagaagagcatcttccgcatcccctggaagcacgcgggcaagcaggactacaaccgcgaggaggacgccgcgctcttcaaggtctccggcctcgggagccggcgggggcgcgccggggagggcccagagacagagcccggggtccccggcgccgcctccgaggcgagcccaggggaccgcgcggggcggacgggcgggcggcggaggcatcaggtggcgtcgccggagccgcaggaggaggaaaggaggcctcggctctcagcgggaccgcgggggccgggagccgggtcctgggcgcgtggaggctgcagggaaaccgctgaaggcccggccgggcccggggaagggcggccaaaggcttgaggggttttgcgcgttcgtccgtgcgttctcgtttccacgcaagcctcccgcccttcctccgggctcccgtctgccgcctccgtccgtgggtccccctcgccctctccgtgcgtccgcgcctgtgccggcggctgttttcgtctctcaccgcgtctctgtttctcttttcgctgcttttctctctgagtctctctctctccatgtttttcctgaggtcagcctctcttctcgctcctgctagctctctgcgggtactcccacctctgtctttctctttgtgtgtctctgtctctctctttcccccatcgcagtggaactcagggcctctgtctagagctgtctcccttgccctttgcgcgagtgcacacacgtgtgtcgttgttacgattgttctcccctaaggcag

SEQ ID NO: 22 - DNA, 23 bp, synthetic construct
  misc_feature 1..23: note = IRF4 probe
  source 1..23: mol_type = other DNA
atcgtacgtaaggttcggagcga

SEQ ID NO: 23 - DNA, 23 bp, synthetic construct
  misc_feature 1..23: note = IRF4 forward primer
  source 1..23: mol_type = other DNA
aaaaaaaaaaaaactccacattt

SEQ ID NO: 24 - DNA, 17 bp, synthetic construct
  misc_feature 1..17: note = IRF4 reverse primer
  misc_feature 7: note = n = acgt
  source 1..17: mol_type = other DNA
tagttgnggagtttggg

SEQ ID NO: 25 - DNA, 2191 bp, synthetic construct
  misc_feature 1..2191: note = BEND4 subregion
  source 1..2191: mol_type = other DNA
caggctgtggcctcgcaaccagcccatctcgctccctgcaggcaggcagtgggctgctttgccgggcagcgcccgcagactcgagataaaggagaggagtcgcggaccccagagtgggtgcctcccacgaggcgtttctgtaaggctcgggccgagatgctcgggaggggcaggaccccgcggcgcggcagcgtgccacggacggggacgaggggatggcggggacgacgacgtgggcggtgggagcagagtgcctgcgactcccggggcaggaaggaggggcgggatggttccccgcgcccgaaatccacggcgtggcggacgcggaggagccccgagtctcacaaccaaggggtgggaaggaaaagggacagagcgagacagagcgcccccgagaaacacaggcgcacaaaaaaagacagaaggaaaaacggaactgagagccagccagcatggactgcgacagcgtgagagtgcatcaaagaggtggcgaagaaagcactagaaggcaaaggagaagtggagagaagaagaaacaaatggaggaagaaggagaaagggaaaaagcagacggaaaaagtgaagtagtacgagggcgtcccagcggggcggcccgagaagctccagcttcttcccgagcggccgccgctatcccccgggggggcgtctggccccactccggaccacgcccgagcgatcctggtcgccgactgccacagccgtgcttcccggcgcgggatccaagccgcggagccacctgttaggcgcgcgccgtcggaagcccaggcgcggcggcgctggagaatcctctcgaagtttccgggtgcgcggggaggccccaggtgcgccccgacatcccgacacggcccagcacgggtaagtgtcggcggccccccgcttctccttcctgggtcccctcccgctgcccccggccgtggcgggaaggaaagttgtgcggagagttggtacctgcgctgagctccaggctggcgctgtcgctacccgtgccgccggtgccggcggccgccgccgcgcctgggccatacctgacgacagcggcgaacgaagacgacgaggaggcggcgggggacgcgggcggcggctgcgccggagtcctcaagtggccctgggatgtggcgggcgtgcaggacggcgacgacgacgaagcggcggcggcggcccggccgggcccgggggggtaggagctctgcgcctggaactgctgcggcggcggctcgctgctgctgatggagacggcggcgtgcggcgcgaagggcggcgggggcggcgggggcgcccgcacgtgcggcagctccaccagggtgggtcgctcgtagcgcttggccagcgccggtctcttgctggggaacgtcttgaggacgctgtaggggctgcgctgcttgtagattttggggacgctgggcccctcctctgccggctgcatctcttcctccatccggcgcctcggggccggtccctcggagcacgtcccctccccgccgggcgccgggctccgagggtgcctccgccgcctgcccgccgggtctgccctggtgcgcgcgtgtgggagggtgtgtgtctgtgccgtggccgccgccgccgccgcctgtcgctgaggctggcatcgccgagcccccgcgcggggggctgccgcccgagctcctgattgacaggctgcctcgccaatgcctggagggagaaaggaggtaaagagcaagtgtttagggtaatatctgctaatgataatgggggcggggcggggcctggcgccgcagccgcccgcggggtctgcctggcggctccgcgcctccgacggggagcgggggaagggggaaagcgaggacctggaggacgcccgggaactggtgaagaaggtggggatccgggatctggctacggcgagactttagagacccagatgtggactcgaggcttctgcggctgcgggcggggtccggcttccgaaacgagctcgtggcgccccctgcatgaccccaaactctcggggttgcacagaggaggggctagtcgttggggcggggtcgtcagagtacgtgtgtattacagcaagttcttctaccaatcgggaattgctctccgatccttctgaaaagaacctcttgaagatcttggcccgggtggtcgcgcggtgtttacggggctttggggtcctgctttccccgagcatcgc

SEQ ID NO: 26 - DNA, 17 bp, synthetic construct
  misc_feature 1..17: note = BEND4 probe
  source 1..17: mol_type = other DNA
taggacggcgacgacga

SEQ ID NO: 27 - DNA, 22 bp, synthetic construct
  misc_feature 1..22: note = BEND4 forward primer
  source 1..22: mol_type = other DNA
agtttttaagtggttttgggat

SEQ ID NO: 28 - DNA, 19 bp, synthetic construct
  misc_feature 1..19: note = BEND4 reverse primer
  source 1..19: mol_type = other DNA
ccaaacgcaaaactcctac

SEQ ID NO: 29 - DNA, 18 bp, synthetic construct
  misc_feature 1..18: note = SEPT9(1a) probe
  source 1..18: mol_type = other DNA
ttgttgcggtcgcggacg

SEQ ID NO: 30 - DNA, 20 bp, synthetic construct
  misc_feature 1..20: note = SEPT9(1a) forward primer
  source 1..20: mol_type = other DNA
gtagttggatgggattattt

SEQ ID NO: 31 - DNA, 17 bp, synthetic construct
  misc_feature 1..17: note = SEPT9(1a) reverse primer
  source 1..17: mol_type = other DNA
cacccgcaaaatcctct

SEQ ID NO: 32 - DNA, 764 bp, Homo sapiens
  source 1..764: mol_type = genomic DNA
agtagggaggtgggcaggagccagtgatgacggaatggcaatcacatttgacctctgatctgtttatttcctcctccttgacgtctccatataaatgttacacgggcatccccacactcggatacgcacccacagtggctgattcgggggtaaccgtgtcatttgcttgcaacactggcacctctgccctgcaccccgggagtgagcagtgagtgaggctcgggtctgggcgctggctccgaatcttcgggctgggagagactccaccatctgggggcggcctgggggagcagccttagtgtcttcctgctgatgcaatccgctaggtcgcgagtctccgccgcgagagggccggtctgcaatccagcccgccacgtgtactcgccgccgcctcgggcactgccccaggtcttgctgcagccgggaccgcgctctgcagccgcagacccggtccacacggccaggggctacgacccttgggatctgccctccgctcagctcgagcttccctcgtggccgacggaacaatgaaggtaactacttatggttttgtccgtgttttacaaaaatgtgtgcgtgaatcgaaccggcgatttctccaagaaacatagttggcagggaggggaggaaggcgagacaaccatggcttatatcccccgcaaacgtctcagtatcttctttatcaatcgtagtttgcggggaccgtgcattctgttcagatttcggtttaacctccactcgcaggacgtgccttctcggacttt

SEQ ID NO: 33 - DNA, 17 bp, synthetic construct
  misc_feature 1..17: note = BCAT1 probe 1
  source 1..17: mol_type = other DNA
tcggttttttcgcggcg

SEQ ID NO: 34 - DNA, 15 bp, synthetic construct
  misc_feature 1..15: note = BCAT1 forward primer 1
  source 1..15: mol_type = other DNA
tacgtggcgggttgg

SEQ ID NO: 35 - DNA, 23 bp, synthetic construct
  misc_feature 1..23: note = BCAT1 reverse primer 1
  source 1..23: mol_type = other DNA
aaaaaaacaaccttaatatcttc

SEQ ID NO: 36 - DNA, 21 bp, synthetic construct
  misc_feature 1..21: note = BCAT1 probe 1a
  source 1..21: mol_type = other DNA
ttcgtcgcgagagggtcggtt

SEQ ID NO: 37 - DNA, 29 bp, synthetic construct
  misc_feature 1..29: note = BCAT1 forward primer 1a
  source 1..29: mol_type = other DNA
gtttttttgttgatgtaattcgttaggtc

SEQ ID NO: 38 - DNA, 20 bp, synthetic construct
  misc_feature 1..20: note = BCAT1 reverse primer 1a
  source 1..20: mol_type = other DNA
caatacccgaaacgacgacg

SEQ ID NO: 39 - DNA, 750 bp, Homo sapiens
  source 1..750: mol_type = genomic DNA
tcaatgagctgttgggtacacctcccagacggggtggcggccgggcagaggggctcctcacttcccagaaggggtggcctggcagaggcacccccaacctccctcccggacggggcggctggccaggcgggggctgcccccaacttcccagacggggtggctgctgggcggaggggctctttacttctcagatggggcggctgccgggtggaggggctcctcacttctcagacggggcggccgggcagaggcgctcctcacctcccagacggggcagcagggcagaggcgctccccacatctcagacgatgggcggccgggcagagacgctcctcacttcctagacgggatggcagccgggaagaggcgctcctcacttcccagactgggcagccaggcagaggggctcctcacatcccagacgatgggcagccaggcagagaagctcctcacttcccagatggggtggcggccgggcagaggctgcaatctcggcactttgggaggccaaggcaggcggctgggaggtggaggttgtagcgagccgagatcacgccactacactccagcttgggcaacattgagcactgagtgaacgagactccgtctgcaatcccggcacctcgggaggccgaggctggcagatcactcccggttaggagctggagaccagcccggccaacacagcgaaaccccgtctccaccaaaaaaatacgaaaaccagtcaggcatggtggcgcgcgcctgcaa

SEQ ID NO: 40 - DNA, 18 bp, synthetic construct
  misc_feature 1..18: note = BCAT1 probe 2
  source 1..18: mol_type = other DNA
ttagacgatgggcggtcg

SEQ ID NO: 41 - DNA, 23 bp, synthetic construct
  misc_feature 1..23: note = BCAT1 forward primer 2
  source 1..23: mol_type = other DNA
tagggtagaggcgttttttatat

SEQ ID NO: 42 - DNA, 20 bp, synthetic construct
  misc_feature 1..20: note = BCAT1 reverse primer 2
  source 1..20: mol_type = other DNA
ccgactaccatcccgtctaa

SEQ ID NO: 43 - DNA, 1531 bp, Homo sapiens
  source 1..1531: mol_type = genomic DNA
ttagccttgaccgaggggcgcttcccggccattcacctagaggttgtttaataaacaaggatgctcgcgaaatatctgcgcttggaaaggcgctcgttcgtggcgcgcattctcgggcctccgcaagcgaccccggtgacagggacaaccgcttcggttttagcgactgcagacagactgggacgagacggttggaggctcctccccaagggatgctggaggggttgcgtcgtaccctgcgcctggccctggcgcgcggccccaggtcgtggtacccagcgccctatgggccgtgcgccggggcttggccacaccgcctgctttcgcttccagccgcgcgctccgtgccactgccgctctctgcagccccgcgtccccgcagcctccccatggccagcccgcttcgctccgctgcggcccttgcccgccaggtacctcgaacccgggcgtttgcggaaggggggaggattggaacccgggtctcggtagctcgcgggcctggccgggcgccttgtcgccgtttcctgcaccatcctccttcgccttgccctccattccgcctccagcgaggcgtcttcccttccccgcatccctgcccgaaatctggagtcccagcctgcaatctccacctcttcgaggttcccgctgcccaggtctagcaccctcatgggtaacccgctccggagcgtggcgaggaccgccacgggggacgtgagggtagctatggactcgctctgagggaggaggcgggagctgaatctctgggctgccagaacccacagccacatcctacgtgactctgccaccccaaaatattttgaccgcagccttctgcctccttggatctcttccttccccacccccacccccgtagttatttagcagattacgcattaaaacaaatgtctgcaggttttcccaattagtcccgcttccctgtgtctttatcttttaaattgcccactaataccatgaggtttaaggtgtggggtggatgctgcggcatcggaggaccctgctggtggaggaaatggttcacgcccgtccccgttccctttgcaggcttgctattgtgcgtctgtgattgacaagaccacgaggctgagcgcgccctggagatttttctataaatggcttaacaccccagtctagactatttgctcggatataagggagacaattgtttttttgttctttgccggcgaaccctggctctgtagggctgacctggaatttaaccagtcttccctgagccggcggaggaggacaaaaaccgccgcgaccccggcagggtgggaagtgcagggcagcgctcccaagacacgcttgttggaggttcgggcctgggtgcttggttgtctgagcctccttttttgtgtttgcctgggtcctggagaggagcgcacggtatcatggtgagcgtcacgtaggttaccccgggtcccgcttacccacctgcatttacttaatggtggtttaattcttctttaaggattgcagtaacggatgctccgcagagtgtaccggagaa

SEQ ID NO: 44 - DNA, 20 bp, synthetic construct
  misc_feature 1..20: note = BCAT1 probe 3
  source 1..20: mol_type = other DNA
tgcgtcgtattttgcgtttg

SEQ ID NO: 45 - DNA, 20 bp, synthetic construct
  misc_feature 1..20: note = BCAT1 forward primer 3
  source 1..20: mol_type = other DNA
ttgggacgagacggttggag

SEQ ID NO: 46 - DNA, 23 bp, synthetic construct
  misc_feature 1..23: note = BCAT1 reverse primer 3
  source 1..23: mol_type = other DNA
aaaacgctaaataccacgaccta

SEQ ID NO: 47 - DNA, 27 bp, synthetic construct
  misc_feature 1..27: note = IKZF1 probe 1a
  source 1..27: mol_type = other DNA
tttgtatcggagtagcgattcgggagg

SEQ ID NO: 48 - DNA, 24 bp, synthetic construct
  misc_feature 1..24: note = IKZF1 forward primer 1a
  source 1..24: mol_type = other DNA
gacgacgtatttttttcgtgtttc

SEQ ID NO: 49 - DNA, 16 bp, synthetic construct
  misc_feature 1..16: note = IKZF1 reverse primer 1a
  source 1..16: mol_type = other DNA
gcgcacctctcgaccg

SEQ ID NO: 50 - DNA, 414 bp, Homo sapiens
  source 1..414: mol_type = genomic DNA
tatcaaacctgcagccggtggaagtcaccaggcccccgtgggaaacaactttctcgtagcatcgtcctcatgtccccacgctgagtttagttctcaccagctctcctctctccgtcccaggagaacggcccttccagtgcaatcagtgcggggcctcattcacccagaagggcaacctgctccggcacatcaagctgcattccggggagaagcccttcaaatgccacctctgcaactacgcctgccgccggagggacgccctcactggccacctgaggacgcactccggtaggtcccctggatgcagtccggggctgtctgggtgtcccgggattcctccactctgcccgcctgggtcccggattgtgtccttgctggctaaccctgagtccctcccagctcgcagtcctgcat

SEQ ID NO: 51 - DNA, 19 bp, synthetic construct
  misc_feature 1..19: note = IKZF1 probe 2
  source 1..19: mol_type = other DNA
tacgtttgtcgtcggaggg

SEQ ID NO: 52 - DNA, 21 bp, synthetic construct
  misc_feature 1..21: note = IKZF1 forward primer 2
  source 1..21: mol_type = other DNA
gttgtatttcggggagaagtt

SEQ ID NO: 53 - DNA, 20 bp, synthetic construct
  misc_feature 1..20: note = IKZF1 reverse primer 2
  source 1..20: mol_type = other DNA
acctaccgaaatacgtcctc

SEQ ID NO: 54 - DNA, 1725 bp, Homo sapiens
  source 1..1725: mol_type = genomic DNA
atgggtaggtcctggctcggtgtcccctagacagacgcatgggccttcccccagcccgtcagtatggtgcaggtgtgatgtgtccgcaggtgtgtgtgtatgtgtgcaggtgtggggtccgcaggcgtgctgggcccccaggccgtgttccccttcccctccccggttgtagatttcagctgttgctgccagacctgaccggttccggaggtggccgcgccccactcactgtcgcctgctttccacaggggacaagggcctgtccgacacgccctacgacagcagcgccagctacgagaaggagaacgaaatgatgaagtcccacgtgatggaccaagccatcaacaacgccatcaactacctgggggccgagtccctgcgcccgctggtgcagacgcccccgggcggttccgaggtggtcccggtcatcagcccgatgtaccagctgcacaagccgctcgcggagggcaccccgcgctccaaccactcggcccaggacagcgccgtggagaacctgctgctgctctccaaggccaagttggtgccctcggagcgcgaggcgtccccgagcaacagctgccaagactccacggacaccgagagcaacaacgaggagcagcgcagcggtctcatctacctgaccaaccacatcgccccgcacgcgcgcaacgggctgtcgctcaaggaggagcaccgcgcctacgacctgctgcgcgccgcctccgagaactcgcaggacgcgctccgcgtggtcagcaccagcggggagcagatgaaggtgtacaagtgcgaacactgccgggtgctcttcctggatcacgtcatgtacaccatccacatgggctgccacggcttccgtgatccttttgagtgcaacatgtgcggctaccacagccaggaccggtacgagttctcgtcgcacataacgcgaggggagcaccgcttccacatgagctaaagccctcccgcgcccccaccccagaccccgagccaccccaggaaaagcacaaggactgccgccttctcgctcccgccagcagcatagactggactggaccagacaatgttgtgtttggatttgtaactgttttttgttttttgtttgagttggttgattggggtttgatttgcttttgaaaagatttttatttttagaggcagggctgcattgggagcatccagaactgctaccttcctagatgtttccccagaccgctggctgagattccctcacctgtcgcttcctagaatccccttctccaaacgattagtctaaattttcagagagaaatagataaaacacgccacagcctgggaaggagcgtgctctaccctgtgctaagcacggggttcgcgcaccaggtgtctttttccagtccccagaagcagagagcacagcccctgctgtgtgggtctgcaggtgagcagacaggacaggtgtgccgccacccaagtgccaagacacagcagggccaacaacctgtgcccaggccagcttcgagctacatgcatctagggcggagaggctgcacttgtgagagaaaatactatttcaagtcatattctgcgtaggaaaatgaattggttggggaaagtcgtgtctgtcagactgccctgggtggagggagacgccgggctagagcctttgggatcgtcctggattcactggctttgcggaggctgctcagatggcctgagcctcccgaggcttgctgccccgtagga

SEQ ID NO: 55 - DNA, 19 bp, synthetic construct
  misc_feature 1..19: note = IKZF1 probe 3
  source 1..19: mol_type = other DNA
tgttttcggagcgcgaggc

SEQ ID NO: 56 - DNA, 21 bp, synthetic construct
  misc_feature 1..21: note = IKZF1 forward primer 3
  source 1..21: mol_type = other DNA
atagcgtcgtggagaatttgt

SEQ ID NO: 57 - DNA, 23 bp, synthetic construct
  misc_feature 1..23: note = IKZF1 reverse primer 3
  source 1..23: mol_type = other DNA
ctcgttattactctcgatatccg

SEQ ID NO: 58 - DNA, 552 bp, Homo sapiens
  source 1..552: mol_type = genomic DNA
gcggcagccgccgccgagccggccggggcgcacggagagcgcgcgggactcgctgcagcggcggccgggtcgcggcgcacccgggccgggaccggagccgagcctagcgcggcgcccgcgacccgtcagccgcggctcctgctccctcgatcccgcgcggggaaagggccggcggctgttggcgtcggcggggcgcggaggaaccgcggcggcggcggcggcggccgcatccttgccgcccgccccggcccagccgcgtcccggagccgtcgggcatggagccgtggaagcagtgcgcgcagtggctcatccattgcaaggtgctgcccaccaaccaccgggtgacctgggactcggctcaggtgttcgaccttgcgcagaccctccgcgatggagtcctgctctgccagctgcttaacaacctccgggcgcactccatcaacctgaaggagatcaacctgaggccgcagatgtcccaggtgaggaggccggcacgggcgccccgcctccagccggcagctcccattaatcatgcggctaatttctttgtgt

SEQ ID NO: 59 - DNA, 18 bp, synthetic construct
  misc_feature 1..18: note = VAV3 probe 1
  source 1..18: mol_type = other DNA
tttcgatttcgcgcgggg

SEQ ID NO: 60 - DNA, 15 bp, synthetic construct
  misc_feature 1..15: note = VAV3 forward primer 1
  source 1..15: mol_type = other DNA
cggagtcgagtttag

SEQ ID NO: 61 - DNA, 14 bp, synthetic construct
  misc_feature 1..14: note = VAV3 reverse primer 1
  source 1..14: mol_type = other DNA
accgccgacccttt

SEQ ID NO: 62 - DNA, 20 bp, synthetic construct
  misc_feature 1..20: note = VAV3 probe 1a
  source 1..20: mol_type = other DNA
cgcggcgttcgcgattcgtt

SEQ ID NO: 63 - DNA, 18 bp, synthetic construct
  misc_feature 1..18: note = VAV3 forward primer 1a
  source 1..18: mol_type = other DNA
cgcgggattcgttgtagc

SEQ ID NO: 64 - DNA, 21 bp, synthetic construct
  misc_feature 1..21: note = VAV3 reverse primer 1a
  source 1..21: mol_type = other DNA
aacaaaaaccgcgactaacga

SEQ ID NO: 65 - DNA, 26 bp, synthetic construct
  misc_feature 1..26: note = IRF4 probe 1a
  source 1..26: mol_type = other DNA
tcgtttagtttgtggcgatttcgtcg

SEQ ID NO: 66 - DNA, 20 bp, synthetic construct
  misc_feature 1..20: note = IRF4 forward primer 1a
  source 1..20: mol_type = other DNA
tgggtgttttggacggtttc

SEQ ID NO: 67 - DNA, 15 bp, synthetic construct
  misc_feature 1..15: note = IRF4 reverse primer 1a
  source 1..15: mol_type = other DNA
cgcctaccctccgcg

SEQ ID NO: 68 - DNA, 20 bp, synthetic construct
  misc_feature 1..20: note = IRF4 probe 1b
  source 1..20: mol_type = other DNA
tacgggggatttcgcgcgta

SEQ ID NO: 69 - DNA, 20 bp, synthetic construct
  misc_feature 1..20: note = IRF4 forward primer 1b
  source 1..20: mol_type = other DNA
ataagtggcgtagacgcggg

SEQ ID NO: 70 - DNA, 20 bp, synthetic construct
  misc_feature 1..20: note = IRF4 reverse primer 1b
  source 1..20: mol_type = other DNA
cctccgctctcccgaaccta

SEQ ID NO: 71 - DNA, 569 bp, Homo sapiens
  source 1..569: mol_type = genomic DNA
gtctgtggatctctgggggagacaagggcacgctgtgtttcccaggcctccttgacgcgggaaccttttgttcccccacgggacatgtgggacactagagttccaccacaggtgcttggctctgtggagtcgttggcctcgaggtggtgtccttggcccccagcactgactccggagctctgtgtttgcagactgccggctgcacatctgcctgtactaccgggaaatcctcgtgaaggagctgaccacgtccagccccgagggctgccggatctcccatggacatacgtatgacgccagcaacctggaccaggtcctgttcccctacccagaggacaatggccagaggaaaaacattgagaagctgctgagccacctggagaggggcgtggtcctctggatggcccccgacgggctctatgcgaaaagactgtgccagagcaggatctactgggacgggcccctggcgctgtgcaacgaccggcccaacaaactggagagagaccagacctgcaagctctttgacacacagcagttcttgtcaggtaaggcacctcgttatctgttag

SEQ ID NO: 72 - DNA, 21 bp, synthetic construct
  misc_feature 1..21: note = IRF4 probe 2
  source 1..21: mol_type = other DNA
tggcgttgtgtaacgatcggt

SEQ ID NO: 73 - DNA, 21 bp, synthetic construct
  misc_feature 1..21: note = IRF4 forward primer 2
  source 1..21: mol_type = other DNA
cgacgggttttatgcgaaaag

SEQ ID NO: 74 - DNA, 25 bp, synthetic construct
  misc_feature 1..25: note = IRF4 reverse primer 2
  source 1..25: mol_type = other DNA
aaacttacaaatctaatctctctcc

SEQ ID NO: 75 - DNA, 19 bp, synthetic construct
  misc_feature 1..19: note = B4GALNT1 probe 1a
  source 1..19: mol_type = other DNA
ttagtcgcgttcgcgtcgt

SEQ ID NO: 76 - DNA, 22 bp, synthetic construct
  misc_feature 1..22: note = B4GALNT1 forward primer 1a
  source 1..22: mol_type = other DNA
ggtttagcggcgttcgttttag

SEQ ID NO: 77 - DNA, 23 bp, synthetic construct
  misc_feature 1..23: note = B4GALNT1 reverse primer 1a
  source 1..23: mol_type = other DNA
aaataaacgacgacttcgtcttc

SEQ ID NO: 78 - DNA, 1600 bp, synthetic construct
  misc_feature 1..1600: note = B4GALNT1 subregion 2
  source 1..1600: mol_type = other DNA
acgagcaggcaatggaatggatgtcgtgggagcaggcggttgagatgccagtgtttggaggctaaggactgggggctgtgagcgaggaccttcccgcgtttgctccgcgcccccgcagtttcctccgcgcccactagaaggcgccggggcgctcgcattccccgcgcggagccgaagcagccgcaacgagccgggagctgagccgcgctgcgctgcggtgcgaagagccgggcggcggccagagccctccccgcgctgccagtgggacgcggagccagggatccccggctttgccccggggctggggtgcaacagactcttaacttggtcctcgcgccccgccaaccgcccccgggcaggaaacgcccagaaccaccaccgcgccgcgctccacaaaagccccgggagttccaagacgggagggatcgggcgcgctccagaggcaggagggtcccccacaccctcaggctcatgcccagctcccccatcgggcagcccccagccccatgaggaccctcaggccggggcgagagcccggcacagcccggaccgaaattttgccgctgccttagagcgttagacaggtcagtgcccgggggtgggtgggggtgggattggttggtgaggggaggaggaggaggcgggaggaggcgggaggaggcgcgcttcccggtccactctgtcccccgcgccgcttgccgaggccactcatcgggtcacctccgccgggggcgcccgccagcacgggcatgattctgcattttttcctgacaggctaggtgtggagccgccctccgcagcccaccccggcccaggtgatgctcagactgaggagtcgggggcgcgccggccagggcgggcggcgggcttggggactgccactgccctgatagagcggggcttttccgcttacgcacggccgcgtcgaaaccgcggcatccaaatgtcttcagcattaagatgccaggcctcgggtgtgtgaggaaaccgagatgcaggagagggcgagaagaaaggaggccgggagaccctggggcctgggaagtgaggggaggggtaccgggaaaaccgcggctggcagtgcaaaccctagcgcgatgtgtggagtggagagcgctcttgggagccggcaggagcctctgaggacgcgggggccaagggccccatcccttgccctcccttcttccctccctttctcactccccaccctacccccacctaggatgtggctgggccgccgggccctgtgcgctctggtccttctgctcgcctgcgcctcgctggggctcctgtacgcgagcacccgggacgcgcccggcctccggctacctcttgcgccgtgggcgcccccgcaaagcccccgcaggcccgagctgccagatcttgctcctgagccccgctacgcacacatcccggtcaggatcaaggagcaagtagtggggtgagtgccgaccgcggcggcgcagcgcagcgctcgctgggggtggtctgggggcttttgttttctccactgctgggctcagatgcctgcattctcctaacgggctgtgtggagtgaagtgggaggtggaagtgggaggctgctgaggcttgggctggg

SEQ ID NO: 79 - DNA, 22 bp, synthetic construct
  misc_feature 1..22: note = B4GALNT1 probe 2
  source 1..22: mol_type = other DNA
cgatgagtggtttcggtaagcg

SEQ ID NO: 80 - DNA, 22 bp, synthetic construct
  misc_feature 1..22: note = B4GALNT1 forward primer 2
  source 1..22: mol_type = other DNA
gaattatgttcgtgttggcggg

SEQ ID NO: 81 - DNA, 22 bp, synthetic construct
  misc_feature 1..22: note = B4GALNT1 reverse primer 2
  source 1..22: mol_type = other DNA
ggatagagtggatcgggaagcg

SEQ ID NO: 82 - DNA, 20 bp, synthetic construct
  misc_feature 1..20: note = GRASP probe 1a
  source 1..20: mol_type = other DNA
tatcgcgcgttcgtcgtgtt

SEQ ID NO: 83 - DNA, 20 bp, synthetic construct
  misc_feature 1..20: note = GRASP forward primer 1a
  source 1..20: mol_type = other DNA
gttgtacgcggcgttggagg

SEQ ID NO: 84 - DNA, 20 bp, synthetic construct
  misc_feature 1..20: note = GRASP reverse primer 1a
  source 1..20: mol_type = other DNA
acgcacctttcgacgaaaca

SEQ ID NO: 85 - DNA, 2248 bp, synthetic construct
  misc_feature 1..2248: note = GRASP subregion 2
  source 1..2248: mol_type = other DNA
gagacggagtctcgctctgtcgcccaggctggagtgcagtggcgcgatctcggctcactgcaagctccgcctcccgggttcacgccattctcctgcctcagcctcccgagtagctgggactacaggcgcctgctaccacgcccggctaattttttgtatttttagtagagacggggtttcaccgtgttagccaggatggtctcgatctcctgacctcgtgatccgcccgcctcggcctcccaaagtgctgggattacaggcgtgagccaccgcgcccggccggacagaacttcttgagggcagagtgagggtgttgggtgtgtgaggtccccaccctttggctggggtgctgggcgtggacaacctggtagtcactacaggcccacaagaatggctgtggttctgtgtgtttggatcgagtatgagagatgtcagaggagatctacagagaaccatgaggagttggaggagggagttcaggagtattccctggagttactacccacccttctcccctttctggctaaggtaggaggctggtattctagcatgccccatggagcaaatctaacccccttgtctgcctggcaggggacaccatcgccagcgtcaatggcctgaatgtggaaggcatccggcatcgagagattgtggacatcattaaggcgtcaggcaatgttctcaggtatgtctgggagccgaggtgcctgaattcctgagctcagcctcttggtatttcctcagcctgtggctcactcaggctttgattctccaacctcagactggaaactctatatgggacatcaattcggaaggcagaactggaggctcgtctgcagtacctgaaggtaggggaacctagataacgtccagcctccaccctcctcttcccaagcctctgccctgtggggggtcacttacagctgaatctcctgtaactgaagatttcttttgtctactccctgatccctcgtctgtacccacgtcctgctagtttcctgctagcttgtgacagtggggtggggactgtctcttgcagcaaaccctgtatgagaagtggggagagtacaggtccctaatggtgcaggagcagcggctggtgcatggtgagtagatcccggggtgtgaggggccacttgttctgctacagacaccccatctgcgcttccccctcagaactggcgggttctagtaaagaacggtttactagtaaacctccacagtaaagcaaggtttgttgagctactactactttgggtactgccgcagccacatttctggttattctcacactagccctctgcaggtaagtaacagatagtgtcatcttcactttacagaggggaacaccagggctcaaagagtttgtgtcaattatttccgaggcccgtttgtgctaagcggcccccataaggatctgagtgataattcctgatttgcgggtgagggaagtagggtctcaggtttgtgcctggccagggccacagagatggtcagcaggacggagcggggacgccccgcccatgccctccgaccctttgcagaggccaccacggtccaggcctgacccgccccctacctctcccgtctctgcgcaggcctggtggtgaaggaccccagcatctacgacacgctggagtcggtgcgctcctgcctctacggcgcgggcctgctcccgggctcgctgcccttcgggcctctgctcgccgtgcccgggcgtccccgcggaggcgcccgacgggccaggggcgacgccgacgacgccgtctaccacacgtgcttcttcggggactccgagccgccggcgctgccgcccccgccgcccccggcccgcgccttcggcccgggccccgccgagacccctgccgtggggccgggccctgggccgcgggccgcgctgagccgcagcgccagtgtgcggtgcgcgggccctggcgggggcggaggcgggggcgcgccgggcgcgctctggactgaggctcgcgagcaggccctatgcggccccggcctgcgcaaaaccaagtaccgcagcttccgccggcggctgctcaagttcatccccggactcaaccgctccctggaggaggaggagagccagctgtaggggcgggggcgggcagggaggtatttatttatttattcgcaacagccagcgctaaaagagggggaggccgagccaagaggaccccaggagcccagagcagcgggagagggtccttcctagcctcggcccgccgggtcggttcct

SEQ ID NO: 86 - DNA, 21 bp, synthetic construct
  misc_feature 1..21: note = GRASP probe 2
  source 1..21: mol_type = other DNA
acgatacgttggagtcggtgc

SEQ ID NO: 87 - DNA, 21 bp, synthetic construct
  misc_feature 1..21: note = GRASP forward primer 2
  source 1..21: mol_type = other DNA
tgcgtaggtttggtggtgaag

SEQ ID NO: 88 - DNA, 22 bp, synthetic construct
  misc_feature 1..22: note = GRASP reverse primer 2
  source 1..22: mol_type = other DNA
caacgaacccgaaaacaaaccc

SEQ ID NO: 89 - DNA, 20 bp, synthetic construct
  misc_feature 1..20: note = BEST4 probe 1a
  source 1..20: mol_type = other DNA
taggttcgcgtagcggatga

SEQ ID NO: 90 - DNA, 23 bp, synthetic construct
  misc_feature 1..23: note = BEST4 forward primer 1a
  source 1..23: mol_type = other DNA
gatcgagcgtagtattagtacgg

SEQ ID NO: 91 - DNA, 21 bp, synthetic construct
  misc_feature 1..21: note = BEST4 reverse primer 1a
  source 1..21: mol_type = other DNA
tacacgacgtaaaccaacgaa

SEQ ID NO: 92 - DNA, 675 bp, synthetic construct
  misc_feature 1..675: note = BEST4 subregion 2
  source 1..675: mol_type = other DNA
tcccggtcagctctcagcccggccgtgggaaggagaggagaggaggatccttgtaacttgctggtggcccaggtgtccctgctatccgtggacgaaatgtaccagaaccttccccccgctgagaaggaccagtactgggatgaggaccagccgcagccaccctacactgtggccacggcggccgagtctctgcggccctcattcctgggctccaccttcaacctgcggtgagtggcttgcactgggcctgacccggcacgcgggtcctcgctcagcctctggggcaccgatgcctcggtccttccccgagagccgatcccgcgtccccgctcccgccctgtgccccggctcagcccgccctcccgcccgcagcatgagcgacgaccctgagcagagcctgcaggtggaggcgtcccccggatctggtcggcccgcgcccgccgcgcagaccccgttgctcggccgcttcctgggcgtaggggcgccctccccggccatcagcctccggaacttcggccgcgtgcgaggcaccccccgccccccgcatctgctgcgcttccgggcggaggagggcggcgaccccgaggccgcagcccgcatcgaggaggaatcggcggagtccggggacgaggccctggagccctgaggtctcgcctgcccccgcccggtttcccc

SEQ ID NO: 93 - DNA, 19 bp, synthetic construct
  misc_feature 1..19: note = BEST4 probe 2
  source 1..19: mol_type = other DNA
tcgatgcgggttgcggttt

SEQ ID NO: 94 - DNA, 21 bp, synthetic construct
  misc_feature 1..21: note = BEST4 forward primer 2
  source 1..21: mol_type = other DNA
ggtttcgttttcggatttcgt

SEQ ID NO: 95 - DNA, 21 bp, synthetic construct
  misc_feature 1..21: note = BEST4 reverse primer 2
  source 1..21: mol_type = other DNA
tctactacgcttccgaacgaa

SEQ ID NO: 96 - DNA, 22 bp, synthetic construct
  misc_feature 1..22: note = BEND4 probe 1a
  source 1..22: mol_type = other DNA
tgcgtttcgatatttcgatacg

SEQ ID NO: 97 - DNA, 20 bp, synthetic construct
  misc_feature 1..20: note = BEND4 forward primer 1a
  source 1..20: mol_type = other DNA
tttcgaagttttcgggtgcg

SEQ ID NO: 98 - DNA, 20 bp, synthetic construct
  misc_feature 1..20: note = BEND4 reverse primer 1a
  source 1..20: mol_type = other DNA
cgaaaaaccgccgacactta

SEQ ID NO: 99 - DNA, 11330 bp, synthetic construct
  misc_feature 1..11330: note = intergenic region 2 subregion 1
  source 1..11330: mol_type = other DNA
gaaacagagtctcgcctcgctccgtcgcccaggctggagtgcggcggcgggatctcggctcactgcaacctccacctgccgggttcaagcgattctcctgcctcagcctccccagtagctgggattacaggcacccgccaccacgcccggctaattttttaatttttagtagagatggggtttcgccatgttagccaagctggttttgagaggagagcactcctcatattgtcttatacttaatttcttgtttgctgaaaaagtggaggttgaaagaatgggcagaagtgaaaatcgtggtcagacaaccgggcgccacatttcgggccttgttgttaaaattcaacccctgacctcaccacttgcgctgtctataaattccagacattgtataaaaacgcattatgaaactcccttttctgttctgtttcgttctgattaccggtgcatgcagcccccagtcacgtacccctcgcttgctcaatcgatcatgacctctccctccacccacagcccctttagagttgtgagcctttaaaagggacaggaattacttattcggggagctccgtttctaggacgtgagtcggccgacgctcccaactgaataaagctcttaccttccacaatccggtgtctgagggattttgtctacgacctctcctgctacagtttcaaactcctgacctcaagtgatccgcctccctcggctttgcaaagtgctgggattacaggcgtgaaccaccgcgcccggcccttgttgtttactgtttccctatagtctttttttttttttttttttttttttgagacggagtctcgctctgttgcccaggctggagtgcagtggcacaatctcggttcactgcaacctctgcctcctaggttcaagcgattcttctgccttagcctcccaagtagctgggactacaggcatacaccactatggccagctaatttttgtatttttagtagagacggggtttcaccatattggccaggctggtctcgaactcctgacctcgtgatccgcccgcctcgggctccgaaagtgcagggattacaggagtgagccactgcgcccggcctactgttttccatagtcgtttctgagaaagaaaaagtaacccttttctgctctcagctagagctggtctgataaacacctaggccatgatgttctccggttcaaactaaaaatttcacaacaccaatatcagacaaagctaccctctcaccaagatgaaagaaagactatttcacaatcatatttgagcacaaacagaacactgttcaaaccataatatgatcaaacattcccctttcccagctactaatagtgactgttaattcttttattttttatttttttgagacggagtcttgctctgtcgccaggctggagtgcagtggcgtgatctcggctcactgcagcctctgcctcccgggttcaagcgattctcctgtctcaacctccggagtagctgggactacaggcgcccaccaccacactcagctaatttttgtatttttagtagagacggggtttcaccatattggccaggctggtctcgaactcctgaccttgtgatctgcccgccttggcctctcaaagtgttgggattacaggcgtgagccactgcacctggccttattttttattttattttatttttttgagacagtctctgtcacccaggctggagtgcagggacgtcatctcagctcactgcaacctctgcctcctgggttcaagcgattctcctccctcagcctcttaagtagctgggattacaggcatgcccaaccatgctcggctaacttttgtattgactgttgattctttaccaattatgtgtttagttctgcaaccattcctcccactttctagataaaaatatcgagattcccaggggaagaattgtcccacaatttccccatagtgtttgctgtctcctctgttgcaatgagccaatatactcagatttgactataggtttgttcctgatggttatagactggagcgcctcaacaccgtagagaagatggatgccgttctgattctttgttatttgccttaaactgttctcccagctcccctcccaaaagcttatagaatcttctacctgttcctactattctgaaacttcatgatctattttcatccaccatgctgggtacacagtgtgctctttcaatataggaatgtatattttggaggtatcattccaaagatgtttatgcatatacagttaaaggtatatatttatttcctgcaactaccatcacccttttgatatacttttgctgcataataaaccatcccaagcttattgacttagaataacaataagttattattttgtgaaggcaccaacatttgcccaaagcaagtcacatagccaatcccagattcaaacagaggagaaatagactctcttgatgagagaagctggaaaatataaccaacatttttttctttttctttttttttgagacggagtttcgctcttattgcccaggctggagtgcaatggtgcaatctcagctcaccgcaacctccgcctcccaggttcaagctattctcctgcctgagcttccctagtagctaggattacaggcatgtgccaccacgcctggctaattttgtatttttagtagagacagggtttctccatgttggtcaggctggtctcgaactcctgacctcagtgatccgcctgcctcggcctcacaaagtgctgggattacaggcgtgagccaccgcgcccggccatgacacaaagtttaaaagaaaaatttttaaaaattttttttggtcaggcgtgatggctcacacctataatcccaggactttgggaggccaaagtgggtggatcacgagtttgagaacagcctggccaatatggtaaaaccccatctctactaaaaatacaaaaaaattagtcgggggtggtggtgcgcacatgtggtcccaactactggagagactgaggtgggagaatcacttgaatctgggaggcgaaggttgtagggagccaagattgtgccactgcactccagcctgggcgacagagattcagtctccaagaaaaaaagtttttttacttttatagatattgtcataaggcaccctgtagaacttgtaccaacttatcctccattcacaaggtatattaaccttcccgccgggcgcggtggctgaagcctgtaatcccagcactttgggaggccaaggcgagcggatcacaaggtcagaagatcgagactatcctgactaacacactgaaaccccgtctctactgacaatacaaaaattagcagggcgtggtggcgggcgcctgtagtcccagctactcgggaggctgaggaaggaaaatggcgtgaaccctggaggcggagcttgcagtgagccgagatctgccactacactccagcctgggcgaaaatgcgagactctgtctcaaaaaaaaaaaaaaaaaaaaaaaaaccctctccaacataaactttaggaaaatttaccattagtttgggcacagtggctcaggcctgtaatcccaacactttgggaggctgaggtgggcatatcgcttgagtccaggagtttgggaccaccctaggcaatacagtgagccctcatctctacaaaaagttaaaaaatcagccaagcatgatggcaagcgcctgtagacccagctacttgggaggctaaggtaggaggatcagctgagcctgagggaggtggaggttgcagtgagccaagatcatgatactgccctccatcttgggtgacagagcgagatactgtctctaaaaaaaaaaagaaagaattccttggatatttctccttggtattttccttttgaactttataatcatattgtctagtttgaataaaaaagaaaaaattctttggacagttttatgaaaatcatgttaaattcagacaccaagtaaaggagaggtgctgtctttatgatgttgagtctcctatccaagaatatgatacaccctcggttaatagggaaggaggctgccctaatgcagtggttcccaaacttgaacattccaaactccctagagagcttgttaagtaacagattgttggggccaccctcggggtttctgattccataggtctaaggtggcactcaatagtttgcgtttatctcaagtttccaggtgatactgaagatgattgtcctgggaccacactttgagaataactggtcattttggagatggttggtggactatatgtaagtgagactaaagcatatttacactcttaaaaaataaaaagtactggtaaatgatccttagggaaaggaggtggaagatctgtaggaggagttgaaaaggaatgttcaggccgggagcggtggctcatgcctgtaatcccagcactttaggaggccaaggcgggcagatcacctgagttcaggggttcgagaccagcctggccaacatggtgaaaccctgtctctactaaaaatacaaaaattagctgggcttgatggcggtcgcctgtaatccccagctactcgggaggctgaggagggagaatcgcttgaacccgggaggcggaggttgcagtgagccgagatcggggcactgcactccagcctgggtgacagagcgagactctgtctcaaaaaaaaaaaaaaaaaaaaaaagaatgtctcttgaatggtgccaatcttggcttccacccacctggcaaaccaacttaacctacgccagcaaaagcaacagttaaagctaatttagcaggaacaaatgtaaggcaaacaactccaggctttcgggaacagaaaaaagttctccggtggatcaataactaattcaaagtagtggacccagcactctggagtggcagcctatattcatcaaataagactgcaactgttaactccctactcgctgccctacccgttcgtctttgctcctccttttctttgctcttccgcttctctcctccgcctcctcaacttcttttctagagccctctcctctttttcctgaccttcctaaaatggttgtattttacagccctttgcggctgatgaaggcttcaaaacctaaaaagcaaacagatgctccctaacacctagctgagaatattttaactcactacaaaggcctttcaaaaccccattcaaaatttcccaccaacaagaagagaaccagtatttccctctggagccgtcctaaggctgttctccctggagcagtgtcggagcgattttggactcttctcagagctgctcagcttgtctgccttcgcccagttgagaagcccatcgtggattcgaagtatgtggtcactacagacactagaatccccagattcctcttttcttttttttttcttttttttgagaccgagtgcaatggcgtgatctcggctcaccgcaacctccgtcttccaggttcaagcaattctcctgcctcagcctcccgagtagctgagattacaggcatgcacctccacgcccggctaattttgtatttttagtagagaaggggtttctccgtgttgaggctggtctcgaactcctgacctcaggtgatccgcccacctcggcctcccaaagtactgggattacaggcgtgagccaccgcgcccggcccagattcctcttttcttgatgaatttggggtgaatggagatgatttctggaatcagttaccataaaaggacagtagccgctgtggcgatttagaagttcatgtttccatggtagctaagcgagagggttaaataaaaacacagcgcccaacgtggggctcgaacccacgaccctgagattaagagtctcatgctctaccgactgagctagccgggcactgattactggcgtcttcttatgtggaatcattttccactgacggagcggttgtatgatctaattgcatattattgcgtgtgaaagaagtttcaggacctaggactggtggacacggcagtagccttttcataatagctttttgccatgaaggaattcggggtttagagagcgatgggggctgcagagagccaggaagtctcgcggaggactcgggaatcacgagtcctgcctgaaaccttagtgttttccgcacattccttccactgagggaacctcctcacccacttcagaggagggtgcgaaagagcccaaggaaactcagatgagaggcgcaaagacctctctgcaaagcattttaattctccatcctggaagaggcactgagttccagagtcacaagggaagggttctctcctctgctcaagtgaaggccaaaagaacaaccgtggtcccagctccgtgggcctccatatcgctctaaagcttcccgcctgggctgcttagcaccttggtgggcgagccgcagtgtgagccaactggaactattgttgtttgagacagggtcccgctctgtcgcccaggctggagtgcagtggcgcgatcatagttcattgcagcctctacttcccgggctcaagcgatgctcccacttcaccctccctaagtagctgggaccaaaagcgcccgccaccatcttaaaaattctttttctggccgggggcgatggctcaagcctgtaatcccagcactttgggaggccgaggcgggtggatcacgaggtcaggggttcgagaccagcctgaccaacatagtgaaacctcgtctctactaaagatacaaaaattagctgggcgtggtggcgggcgcctgtaatcccagctactcaggaggctgaggcaggagaattgcttgaacccgggaggcgggggttgcagtgagccgagatcgcgccactgcactccagcctgggcgacagagcaagactctgtctcaaaaaaaaaaaaaaaaaaaaaaattctgacattgtggggaggcgtctcaagctggtcgcgaactcctgggctccagggattctcccgcctccgagacttcccaaagctgctgggattacgtaatggcgcgagccaccacgtcggcctggagctattgttattcaccgaatctgtggactgcacttccgcggggatgccttaagcgaaggcagaattacaagcatgtgtcactcttttaaaagtgttaattaaaaaaaaaaaaaaccgccaccccagcaagttagaaccacctgccgtgactcggattcgaaccgaggttgctgcggccacaacgcagagtactaaccactatacgatcacggcgagccactaaccaggcggcgcgctacagctggatttaatgcctcttgaaataggaatggctatttcgtgctacttttatttggccagtccctgacgtccgcatcaatcaattccaaactttttcactctgcaaccttgaagctccgacacctgaatcagtttcttagactctaaatccctcgatgccagcgatagcaccacccgctccgctgggcggcggcgggccaaggtcctgactagagggcagaaagcgtcagctgcaacccgggaccacgccgcctctcgcctctctcctctcacctctctgcctccatttccctcttccccctccaaggaatcaagctgcttcgcccagggatgagaggggcagcctcgaaggatttttcaaattacatctgcagcctgtaccacggaattgaggtttctcttcccagaatggtggaaccggaagaaaaacggagctagtgagctggggaggggatgagagccccgtcttaatttcttgcttccctcacaggtacaagaagcgctgtgtactctctggcattgtgggagcttgtgctgacttcctcatcttgactcataaatatatcagagccacctctgccgattcagaaaaacaaatccaaccagcctctatttcagacacttccttagacccctaggagagttattgttaacttccctagacccctaggagagttattgtttggacgccagcggccgaacccatcagacgggctaggcgcgcacgtgcagttaccaaaatacagatgtttactgtgggagggacagaccatactggtgcagacctaggacacaaaagtggtcaaaactcttttcctgtgttccctactttgctcggtttccaggcctactcagtctaaaaagctgaagagaaaaactgacactgcgttggccgggaatcgaacccgggtcaactgcttggaaggcagctatgctcaccactataccaccaacgcatctgaaatacacttgattcctttagagtatcagaactaaataatcaggtttgtcttcccgtttatttctaggctaagcaatttagactgcaggaaaaacctacaagaggaaaattaaaaggaagctctctggaatttctcctattaaaaattctgtagtagtatcttgtttcacagctttaagaaaagtcaattctagtttcctggacatttattccacacatgcgcaaaattacatatgtacaagaccgtatatgacagcatttttttttccaaagagcaaagggctagaaataacctaagtgtctataataggaagctggctaaactaattatggaaaatccatacaacggaatgctatgtgccagaagaaagaatgaggaagttcttcatgtctaatctgtaagtacttccaaaatatactgttaaatggaaaaggcaaagtgcagaaagtgtgtatagattacttccatttgtacaagggggagagaatgtttaaatatatatacgtatgtatatatgcatgtacttgcatttgcataaaacatctctaacatcatgaagaaacttaacagcggttacttcattagagagaaaataaatggtagaggtgaaaggtttatcagttctgcccttttgtatatttgaatcctaaaccatgtaaatatattaccttttcgaaaatccagtaattaaattgaaagaaaatacgttactgaaggatatttatttccactgcaaagtgttagaaatacattgttaaccttaaaaatagctggtgttggccgagcatggtagctcacgcctataatcccgtcactttggtaaggcagaggcgggtggatcacctgaggtcaggagttcgagaccggcctcaccaatatggtgaaccccgtctctactacaaatacaaaattagccgggcgtggtagcgcaggcctgtaatcccagctacttgggaggctgaggcaggagaatcgcttgaacccgggaggcggaggttgcagtgagccgagatcgcgccactgcactccagcctggggcaacgacagcgaaactccgtctcaacaacaacaaaaacagctggtgataaaatagtattatagcatacttccactttgtttcaaaacctagatattgagtggtcttcgggtgatagaatggtgagcgatttctttatttgtgtttttctacattttctgtatttcagttttcagtgggatggggaagattgactagcagataacgtttatttaaaagatcctgagagaaagcagtaaaagaagatgttactctttccctgaccgggaatcgaacccgggccgcggcggtgagagcgccgaatcctaaccactagaccaccagggaagctgctaacccttcccggttgcagctatatgattctactaagtgctgcggttcgtgcctgtaactgctaaacactgaagccaaagtggccagattgctggagctcctagttcgagaccagcctgggcaaagtggcaaacccgggctctatcaaaagcacaaaaaaattagccgggcgtggtggcgcttgcctgtagtcccatctacccgagaggccggatcgcttgagcctggtaggcggaggttgcagcgagccgtgatcgtgccactgcactccaacttgatgacagggccagagccttcctcaaaaaaaaaaaaaaattacattattctaactaaaagtttatttccacttattctttttcatattatttttcactgcctagattctgagattcttgcatactgggcctttcctatgttggggcttcttcccggtacttctttcctgcagtagaaaacattgtgaaagaattctccagcccggctctcagagcctagggagcatcgtgtacacgtgattacagtccccaagaccagagaccaatgtccggagagaagagggtgagacagagaggaagctcacctccttgtagttgcagtgatttccgaaattgtgaacattagaaaagtagagacccagctacgtctttgccaaaaacaaccaggaacttttccttaaggaacataaaagacgtcatgcgagtaacactaggagatcctgggcccactgtaccttttttcatgtcgtgtgaattgtaggccaaactgttaaaacaaatattacagacgagtgaaaatcactcagcctagaggtacttggtgctcagcaggatctgagctcaactcactagtgggagactaagagaaactcagggcctttaacctttaaaaattacgaggtcccgggcgcggtggctaatgcctgtaatcccagcactttgcgaggccgaggcgggtggatcacgaggtcaagagatcgagatcattctggccaacatagtgaaaccccgtctctactaaaaatacaaaaagtagccggcgtggtggcgggcgcctgtagtcccagctactcgggaggctgaggcaggagaatcgtttgaacccgggaggcggaggttgcagtgagcggagattgcgccattgcactccagcctgggcatcaagagtgaaactttgtctcaaaaaaaaaaaaaaaaaaaaaaaataaattatgaggaagccgggcgcagtggctcagacgcctgtaatcccaggactttgggaggctgaggcgggtggattacctgaggtcagaagttcgagaccaacctggccaacatggtgaaatcctgtctctactaaaaatacaaaattagccaggcgtggtggcgcttgcctgtaatcccaggactttgggaggctgaggcgggtggattacctgaggtcagaagttcgagaccaacctggccaacatggtgaaatcctgtctctactaaaaatacaaaattagccaggcgtggtggcgcttgcctgtaatcccagctactcgggaggctaaggcaggagactcgctttaacccaggagacggaggttgcagtgagccgagatcacgccattgcaccccagcctgggcaacaagagcaacacaaaataaaaattgcgaggaaggaaaagagggagtgaagagaaagaaaactggggtgcatgcattaatgtgttgcaagctaactttatgagcgagaaaagaaagcaaatgcgggctggatacagtggctcaagcttgtaatc

SEQ ID NO: 100 - DNA, 21 bp, synthetic construct
  misc_feature 1..21: note = intergenic region 2 probe 1
  source 1..21: mol_type = other DNA
cggtgagagcgtcgaatttta

SEQ ID NO: 101 - DNA, 23 bp, synthetic construct
  misc_feature 1..23: note = intergenic region 2 forward primer 1
  source 1..23: mol_type = other DNA
ttattttttttttgatcgggaat

SEQ ID NO: 102 - DNA, 23 bp, synthetic construct
  misc_feature 1..23: note = intergenic region 2 reverse primer 1
  source 1..23: mol_type = other DNA
ataactacaaccgaaaaaaatta

SEQ ID NO: 103 - DNA, 22 bp, synthetic construct
  misc_feature 1..22: note = intergenic region 2 probe 1a
  source 1..22: mol_type = other DNA
cgaggttgttgcggttataacg

SEQ ID NO: 104 - DNA, 21 bp, synthetic construct
  misc_feature 1..21: note = intergenic region 2 forward primer 1a
  source 1..21: mol_type = other DNA
ttgtcgtgattcggattcgaa

SEQ ID NO: 105 - DNA, 20 bp, synthetic construct
  misc_feature 1..20: note = intergenic region 2 reverse primer 1a
  source 1..20: mol_type = other DNA
caactataacgcgccgccta

SEQ ID NO: 106 - DNA, 1020 bp, synthetic construct
  misc_feature 1..1020: note = intergenic region 2 subregion 2
  source 1..1020: mol_type = other DNA
agttcctttgggcctgggccggtggacgtgagcgtgggaaggacaagaacccgcggtgccccccaccgcactatcctcgggtctccagaggtgggatccaccgggcaggggcctttgctggattctaaaccggctctggggatacaagaacagctgcctttgagaaacagttcaggtctctatattccagacttcctagtaggactaaacgcttaacgttcacacgggaattcatggttctcctaaaaccctgcggtggaatgccttccttcaccgagcatttattgggcacctactaggtgctaggctggctctgggcgaagggctgcagcctgtgcaaactccaggtccctgtccggtggatcccacctctgagggcccgagggtgacgcggtgaggacaccacgggttctggtccttcccacgcgcgcgtccgctagcccaggcccggcggaaatgactgtgagctcaaggtgtgaagcggggctaagaatgggaaagcgagtgacttccgccggagaagctgcagttgtcgcctgtagaggggccggcgacttttgagacggtgaagagcaggcgggggaaccagtgaagagcagacggtgaggagcaggcggccgtttggccgttggagtcccccagctgactctgcccgggtagaatgtccaaagtgcccaaagactcgactcttggcttcaatgtctcccgtgttctgggtttctggagtgcgcgggattggacaggctacaaacatatgagattatctacggccagaggttaaaatgccatttctggtatcagcaaatctaaaccattagagtctctgtggcgccatcggttagtgccttcggctgtttgaaccgaaaggctggtggttcaagcccacccagagatggtaccttttacttaggcaagattcacgctttctgtttaaagactttaatcctgggaatcttccggacctctactagctttaaattcgatgccaaaatacgctgtgcgaaggctcaagttccatgg

SEQ ID NO: 107 - DNA, 19 bp, synthetic construct
  misc_feature 1..19: note = intergenic region 2 probe 2
  source 1..19: mol_type = other DNA
ttacgcgcgcgttcgttag

SEQ ID NO: 108 - DNA, 20 bp, synthetic construct
  misc_feature 1..20: note = intergenic region 2 forward primer 2
  source 1..20: mol_type = other DNA
acgcggtgaggatattacgg

SEQ ID NO: 109 - DNA, 22 bp, synthetic construct
  misc_feature 1..22: note = intergenic region 2 reverse primer 2
  source 1..22: mol_type = other DNA
gttcggcggaaatgattgtgag

SEQ ID NO: 110 - DNA, 1300 bp, synthetic construct
  misc_feature 1..1300: note = intergenic region 2 subregion 3
  source 1..1300: mol_type = other DNA
aggtgatccgcctgcctcagcctcccaatatgctgggattacagtcatgagccaccgcgcccggccgacaaaattttcaatgtactaagcgccactgcattgtatacattaaaatagttaaaattgtgaactttatgttgtgtgtattttactacaacaaaaaaataatgaagggggccaggtgcagtggctcatatctgtaatcttagcactttgggaggccgaggcaggcggccgggaggtggaggttgcagtgagctgagatcatgctactgcactctagcctgggcaacattgagcattgagtgagtgagactccatctaaaaaaaaaagaagaagaaaggaaaatcctagcaggattttctacagatacagacaagattattactattactattattattattatttccttcgagatgaggtttcactctgtcacccaggtggagtgcagtggcgggatctcagctcaccacaatctccacctcccaggctcaagcgatcctcccacctcagtctccagagtagctgggaccacaggcgcatgccaccacatccagctaatttttttgtatttttggtagagacaaggtttcaccatgttggccaggctggtcttgaactccggagctcaggcgatccacccacctcggcctcccaaagtgctggaattacagcatgagccaccaccttgttttaaaaatctgtaactttaagacaagagaccgggcgcggtggctcacgcctgtaatcccagcactttgggaggccgaggcgggcggatcacgaggtcaggagatcgagaccatcctggctaacacagtgaaaccctgtctctactaaaaatacaaaaaatcagccgggcgtggtggcgggcgcctgtagtcccaggtactcggaaggctgaggcaggagaatggcgtgaacccgggaggcggagattgcagtgagccgagatcacgccactgcactccagcctgggcgacagagcgagactgcgtctcaaaaaaaaaagacaagattattctaaaagttatatcaaaggcaaagaagcggacatagctaaaacaatttttaaaaataattaaatgaggttgggcgcggtggctgacacctgtaatcccagcactttgggaggccgaggcgggcagatcacttgaggtcaggagttggagaccagcctggccaaaatggcgaaaccccgtctctactaaaaatacaaaaattagccaggcgtggtggtgtgtgcctgtaatcccagctattcggcaggctgaggcaggagaatcacttgagccc

SEQ ID NO: 111 - DNA, 19 bp, synthetic construct
  misc_feature 1..19: note = intergenic region 2 probe 3
  source 1..19: mol_type = other DNA
ttgggaggtcgaggcgggc

SEQ ID NO: 112 - DNA, 20 bp, synthetic construct
  misc_feature 1..20: note = intergenic region 2 forward primer 3
  source 1..20: mol_type = other DNA
gataagagatcgggcgcggt

SEQ ID NO: 113 - DNA, 24 bp, synthetic construct
  misc_feature 1..24: note = intergenic region 2 reverse primer 3
  source 1..24: mol_type = other DNA
ctcgatctcctaacctcgtaatcc

SEQ ID NO: 114 - DNA, 15 bp, synthetic construct
  misc_feature 1..15: note = intergenic region 1 probe 1
  source 1..15: mol_type = other DNA
ttgaggggcggtcgc

SEQ ID NO: 115 - DNA, 19 bp, synthetic construct
  misc_feature 1..19: note = intergenic region 1 forward primer 1
  source 1..19: mol_type = other DNA
gtttcgttaggttggagag

SEQ ID NO: 116 - DNA, 23 bp, synthetic construct
  misc_feature 1..23: note = intergenic region 1 reverse primer 1
  source 1..23: mol_type = other DNA
ctacaaaacaaaacctaaaatcc

SEQ ID NO: 117 - DNA, 20 bp, synthetic construct
  misc_feature 1..20: note = intergenic region 1 probe 1a
  source 1..20: mol_type = other DNA
cgggtttgcggttttcggtc

SEQ ID NO: 118 - DNA, 23 bp, synthetic construct
  misc_feature 1..23: note = intergenic region 1 forward primer 1a
  source 1..23: mol_type = other DNA
cgatcgtaaagagatagcgattt

SEQ ID NO: 119 - DNA, 20 bp, synthetic construct
  misc_feature 1..20: note = intergenic region 1 reverse primer 1a
  source 1..20: mol_type = other DNA
aatcgtcaccgtaacgcgaa

SEQ ID NO: 120 - DNA, 1250 bp, synthetic construct
  misc_feature 1..1250: note = GPAM subregion 1
  source 1..1250: mol_type = other DNA
aatgaagtgaagagaggatgaggagaggacaaagaggctcgtttgtgccaacaggaggtccacgttttgcacttcctccctccgcacagttcgctctaggtcaaggagtaataaagaagcaatatcccagaggcaccagccagcagcatgcgctgagagaagctgactagaggatctgaaaaggacagaggctggaagaccagctgtgaggtttaaatcttccactgcttaccatctgtgtgattttttattaccataagttggttaacttctatgccttagttttcccatctggaaaatgggcagaatgatagctcttaacctcctggattgttgagaggacggaataatataaacaaagggtctaccacagtgtgtaacacacagtgagcgctcagtccaatcaatggtaacgctgtcattaattatctccagcataccggctgctctcagagtaccccttactgcctcaatgttccctagggacccaggcgggctggctggcggcgcctccgcgcgtgcagatacttaggggactgagtccataaggactccttccaacccaggggaacccatgccccagcgcagtctccccaggagagatgaatcctgatccccacccctgcacgagcccgaccgatttctcagggagaagaccggagctcgggtgtcagggaataggggacacgactgccccagcaacttgcaggagtcgcaccacctccatgcacttgtcccggcgctcccggcccgagtagcctcccgcagcccacacctgccctggcagttcgcaccctagcagctccagcttcggctgctgcagaagcccgcacttccagtcccggccaatgccagctgcagtggcgcaccctgatgacgcaaccggcgcgtggcattgacgcggggccgccggctagccagcgccgggggcggggcccggcctgcgagcctcagggagcgtgagcggatccgagggtgtaatgtgtgtactcgagtgtgcgtgcctgtgtgtggctaaagatagtgtgtgagcgcctggacagatggttaccctgcctaggccatgcgtgtgtgagtgtgtgtgggtacctcattctgctttgtgtaaattcagcttatccgggagcttgtccctcttccaggctctgttgggaatgtgcgcgtgggctatcaggttatgtgtgtggtctgactttttatgagatctgtaagactatgtaggatttactacgaatgggagaggcagggat

SEQ ID NO: 121 - DNA, 19 bp, synthetic construct
  misc_feature 1..19: note = GPAM probe 1
  source 1..19: mol_type = other DNA
cgtgagcggattcgagggt

SEQ ID NO: 122 - DNA, 18 bp, synthetic construct
  misc_feature 1..18: note = GPAM forward primer 1
  source 1..18: mol_type = other DNA
ggtttgcgagttttaggg

SEQ ID NO: 123 - DNA, 19 bp, synthetic construct
  misc_feature 1..19: note = GPAM reverse primer 1
  source 1..19: mol_type = other DNA
caaacgctcacacactatc

SEQ ID NO: 124 - DNA, 19 bp, synthetic construct
  misc_feature 1..19: note = GPAM probe 1a
  source 1..19: mol_type = other DNA
atcggcgcgtggtattgac

SEQ ID NO: 125 - DNA, 24 bp, synthetic construct
  misc_feature 1..24: note = GPAM forward primer 1a
  source 1..24: mol_type = other DNA
gttgtagtggcgtattttgatgac

SEQ ID NO: 126 - DNA, 20 bp, synthetic construct
  misc_feature 1..20: note = GPAM reverse primer 1a
  source 1..20: mol_type = other DNA
cgacgctaactaaccgacga

SEQ ID NO: 127 - DNA, 1350 bp, synthetic construct
  misc_feature 1..1350: note = VASH2 subregion 1
  source 1..1350: mol_type = other DNA
gttgcggtggccaatagacgcattcggaacatcggcggctgcccgggtgacttggttatatgtcacagaataacattcgagaatgggacatggaatgaggcgacggccccagcaagccccagcagccccagccccagccccaggcccagcagcagcagcagcagcccctgctctcccgccgcccggagaggctctgcagccatgaagccaaccgtcccgaggtaggatcttggagctgccgcgcgcccttcctgcgcgccgcccgcctgcagccagtccctcccggtgataggcgctggaactcggggaaaagggggcggatggagctctttccactagatccccgccggggtccgggagggcttcctggaagaaagcgggccgccttgcaagccaaggctgctgcagcgccctcgcgccagctctgggcgctcacatgccagcacgttcgtggctcccctcctctcttggccacatctgaggacccaggaatgtgtggagccttgcgggaacctcctgttccttcatgctacacaagctgtctttcttctccccacatcttgcgctccgcatcccccaagctccttgtgcccctccatccccaaccccccgggtttaggtgtgtgtgaagcttcgtggcacattttgagctgcctttctaggtaatcgcagggctggaagcccgtcatcgattctcagggaggctgtcagcgtgcaggggggagcggggagtgtcgtggagacactccgggacccctcactcggttccgctgtgcgtccacttagctgtggtgtcagctgtgtctccgctgatttcaggcaccgccggtaagcagggagcctccgcggagctcccgccgccgctcccccttggtgagtcctgccgcagcgagaggcatggagaaggccgcccccgcggggcgctgatcccctcgccgcgcccgcgcgcacacgccccccgccgccgccgccgctgccgccgccgcgcgcccccagtacctcgctccccgcccaggccccaccatgaccggctccgcggccgacactcaccgctgcccccaccccaaaggcgccaaaggcacccggtcccggagcagccacgcgcggcccgtgagcctcgccaccagcgggggctcagaggaggaggacaaagacggcggggtgctgttccacgtcaacaagagcggcttccccatcgacagccacacctgggagcgcatgtggatgcacgtggccaaggtgcaccctaaggggggagaaatggtgggcgccatcaggaacgccgccttcttggcaaaggtcagtggcttccagggcggagttggggggctgggggtaggtaggcagcga

SEQ ID NO: 128 - DNA, 18 bp, synthetic construct
  misc_feature 1..18: note = VASH2 probe 1
  source 1..18: mol_type = other DNA
ttcggtttcgttgtgcgt

SEQ ID NO: 129 - DNA, 17 bp, synthetic construct
  misc_feature 1..17: note = VASH2 forward primer 1
  source 1..17: mol_type = other DNA
ttagcgtgtagggggga

SEQ ID NO: 130 - DNA, 20 bp, synthetic construct
  misc_feature 1..20: note = VASH2 reverse primer 1
  source 1..20: mol_type = other DNA
cgaaaacacaactaacacca

SEQ ID NO: 131 - DNA, 20 bp, synthetic construct
  misc_feature 1..20: note = VASH2 probe 1a
  source 1..20: mol_type = other DNA
tgtcgcgcgttttttttgcg

SEQ ID NO: 132 - DNA, 20 bp, synthetic construct
  misc_feature 1..20: note = VASH2 forward primer 1a
  source 1..20: mol_type = other DNA
ttcgtcgttcggagaggttt

SEQ ID NO: 133 - DNA, 21 bp, synthetic construct
  misc_feature 1..21: note = VASH2 reverse primer 1a
  source 1..21: mol_type = other DNA
ttccaacgcctatcaccgaaa

SEQ ID NO: 134 - DNA, 30 bp, synthetic construct
  misc_feature 1..30: note = ACTB probe
  source 1..30: mol_type = other DNA
accaccacccaacacacaataacaaacaca

SEQ ID NO: 135 - DNA, 24 bp, synthetic construct
  misc_feature 1..24: note = ACTB forward primer
  source 1..24: mol_type = other DNA
gtgatggaggaggtttagtaagtt

SEQ ID NO: 136 - DNA, 25 bp, synthetic construct
  misc_feature 1..25: note = ACTB reverse primer
  source 1..25: mol_type = other DNA
ccaataaaacctactcctcccttaa

SEQ ID NO: 137 - DNA, 22 bp, synthetic construct
  misc_feature 1..22: note = SDC2 probe
  source 1..22: mol_type = other DNA
ttcggggcgtagttgcgggcgg

SEQ ID NO: 138 - DNA, 24 bp, synthetic construct
  misc_feature 1..24: note = SDC2 forward primer
  source 1..24: mol_type = other DNA
gtagaaattaataagtgagagggc

SEQ ID NO: 139 - DNA, 23 bp, synthetic construct
  misc_feature 1..23: note = SDC2 reverse primer
  source 1..23: mol_type = other DNA
aacgactcaaactcgaaaactcg